European Patent Specification EP 3 638 697 B1, published September 23, 2026. Title: ANTI-IL1RAP ANTIBODIES AND ANTIBODY DRUG CONJUGATES. Applicant: BLUEFIN BIOMEDICINE, INC. The sequence listing filed with the application follows.

SEQUENCE LISTING (286 sequences)

SEQ ID NO: 1 - protein, 114 aa, Artificial Sequence
  Description of Artificial Sequence: Synthetic polypeptide
QVELQESGPGLVKPSDTLSLTCTVTGGSISTYYWSWIRQPPGKGLEWIGYIFYTGTTNYNPSLKSRVTISVDASKNQFSLKLNSVTAADTAVYYCARDGSLDYWGQGALVTVSS

SEQ ID NO: 2 - protein, 10 aa, Artificial Sequence
  Description of Artificial Sequence: Synthetic peptide
GGSISTYYWS

SEQ ID NO: 3 - protein, 16 aa, Artificial Sequence
  Description of Artificial Sequence: Synthetic peptide
YIFYTGTTNYNPSLKS

SEQ ID NO: 4 - protein, 6 aa, Artificial Sequence
  Description of Artificial Sequence: Synthetic peptide
DGSLDY

SEQ ID NO: 5 - protein, 107 aa, Artificial Sequence
  Description of Artificial Sequence: Synthetic polypeptide
DIQMTQSPSSLSASVGDRVTITCRASQSISNYLNWYQQKPGKAPKLLIFVASLLQSGVPSRFSGSGSGTDFTLTISSLQPEDFATYYCQQSYSTPFTFGPGTKLEIK

SEQ ID NO: 6 - protein, 11 aa, Artificial Sequence
  Description of Artificial Sequence: Synthetic peptide
RASQSISNYLN

SEQ ID NO: 7 - protein, 7 aa, Artificial Sequence
  Description of Artificial Sequence: Synthetic peptide
VASLLQS

SEQ ID NO: 8 - protein, 9 aa, Artificial Sequence
  Description of Artificial Sequence: Synthetic peptide
QQSYSTPFT

SEQ ID NO: 9 - protein, 124 aa, Artificial Sequence
  Description of Artificial Sequence: Synthetic polypeptide
QVQLVESGGGVVQPGRSLRISCAASGFTFRSYGMHWVRQAPGKGLEWVAIIWHDESYKYYVDSVKGRFTISRDNSKNTLYLQMNSLRAEDTAVYYCARGDYYGSGSYYDAFDIWGQGTMVTVSS

SEQ ID NO: 10 - protein, 10 aa, Artificial Sequence
  Description of Artificial Sequence: Synthetic peptide
GFTFRSYGMH

SEQ ID NO: 11 - protein, 17 aa, Artificial Sequence
  Description of Artificial Sequence: Synthetic peptide
IIWHDESYKYYVDSVKG

SEQ ID NO: 12 - protein, 15 aa, Artificial Sequence
  Description of Artificial Sequence: Synthetic peptide
GDYYGSGSYYDAFDI

SEQ ID NO: 13 - protein, 107 aa, Artificial Sequence
  Description of Artificial Sequence: Synthetic polypeptide
DIQMTQSPSSLSASVGDRVIITCRASQGISNYLAWFQQKPGKCPNLLIYAASTLRSGVPSRFSGSGSGTDFTLTISSLQPEDVATYYCQKYNSAPYTFGQGTKVEIK

SEQ ID NO: 14 - protein, 11 aa, Artificial Sequence
  Description of Artificial Sequence: Synthetic peptide
RASQGISNYLA

SEQ ID NO: 15 - protein, 7 aa, Artificial Sequence
  Description of Artificial Sequence: Synthetic peptide
AASTLRS

SEQ ID NO: 16 - protein, 9 aa, Artificial Sequence
  Description of Artificial Sequence: Synthetic peptide
QKYNSAPYT

SEQ ID NO: 17 - protein, 121 aa, Artificial Sequence
  Description of Artificial Sequence: Synthetic polypeptide
QVQLVESGGGVVQPGRSLRLSCAASGFTFSHYGMHWVRQAPGKGLEWVAVIWYDGSKKYYVDSVKGRFTISRDNSKNTLYLQMNSLRGEDTAVYYCARDGGAVADNWIDSWGQGTLVTVSS

SEQ ID NO: 18 - protein, 10 aa, Artificial Sequence
  Description of Artificial Sequence: Synthetic peptide
GFTFSHYGMH

SEQ ID NO: 19 - protein, 16 aa, Artificial Sequence
  Description of Artificial Sequence: Synthetic peptide
IWYDGSKKYYVDSVKG

SEQ ID NO: 20 - protein, 12 aa, Artificial Sequence
  Description of Artificial Sequence: Synthetic peptide
DGGAVADNWIDS

SEQ ID NO: 21 - protein, 107 aa, Artificial Sequence
  Description of Artificial Sequence: Synthetic polypeptide
DIQMTQSPSSLSASVGDRVTITCRASQSIRSYLNWYQQKPGKAPKLLIFAASSLQSGVPSRFSGSGSGTDFTLTVSSLQPEDFATYSCQQSYSTPYTFGQGTKVEIK

SEQ ID NO: 22 - protein, 11 aa, Artificial Sequence
  Description of Artificial Sequence: Synthetic peptide
RASQSIRSYLN

SEQ ID NO: 23 - protein, 7 aa, Artificial Sequence
  Description of Artificial Sequence: Synthetic peptide
AASSLQS

SEQ ID NO: 24 - protein, 9 aa, Artificial Sequence
  Description of Artificial Sequence: Synthetic peptide
QQSYSTPYT

SEQ ID NO: 25 - protein, 120 aa, Artificial Sequence
  Description of Artificial Sequence: Synthetic polypeptide
QVQLVESGGGVVQPGGSLRLSCAASGFTFSSHGMHWVRQAPGKGLEWVAVIWYDGSNKFYTDSVQGRFTISRDNSKNTLNLQMNSLRAEDTAVYYCAREGLRAGYYFDFWGQGTLVTVSS

SEQ ID NO: 26 - protein, 10 aa, Artificial Sequence
  Description of Artificial Sequence: Synthetic peptide
GFTFSSHGMH

SEQ ID NO: 27 - protein, 17 aa, Artificial Sequence
  Description of Artificial Sequence: Synthetic peptide
VIWYDGSNKFYTDSVQG

SEQ ID NO: 28 - protein, 11 aa, Artificial Sequence
  Description of Artificial Sequence: Synthetic peptide
EGLRAGYYFDF

SEQ ID NO: 29 - protein, 107 aa, Artificial Sequence
  Description of Artificial Sequence: Synthetic polypeptide
DIQMTQSPSSLSASVGDRVTITCRASQRISFYSNWYQQKPGKAPKLLIYAASSLQSGVPSRFSGSGSGTDFTLTISSLQPEDFATYFCQQSHSTPLTFGGGTKLEIK

SEQ ID NO: 30 - protein, 11 aa, Artificial Sequence
  Description of Artificial Sequence: Synthetic peptide
RASQRISFYSN

SEQ ID NO: 31 - protein, 9 aa, Artificial Sequence
  Description of Artificial Sequence: Synthetic peptide
QQSHSTPLT

SEQ ID NO: 32 - protein, 120 aa, Artificial Sequence
  Description of Artificial Sequence: Synthetic polypeptide
QVQLVESGGGVVQPGRSLRLSCAASGFTFRNYGIHWVRQAPGKGLEWVAVIWYDGSNKFYADSVKGRFTISRDNSKNTLYLQMNSLRVEDTAVYYCAREEGIAVAPFDYWGQGTLVTVSS

SEQ ID NO: 33 - protein, 10 aa, Artificial Sequence
  Description of Artificial Sequence: Synthetic peptide
GFTFRNYGIH

SEQ ID NO: 34 - protein, 17 aa, Artificial Sequence
  Description of Artificial Sequence: Synthetic peptide
VIWYDGSNKFYADSVKG

SEQ ID NO: 35 - protein, 11 aa, Artificial Sequence
  Description of Artificial Sequence: Synthetic peptide
EEGIAVAPFDY

SEQ ID NO: 36 - protein, 107 aa, Artificial Sequence
  Description of Artificial Sequence: Synthetic polypeptide
DIQMTQSPSSLSASVGDRVAITCRANQSIASYLNWYQQKPGKAPKLLIYGASSLQNGVPSRFSGSGSRTDFTLTISSLQPEDFATYYCQQSYSTEITFGQGTRLEIK

SEQ ID NO: 37 - protein, 11 aa, Artificial Sequence
  Description of Artificial Sequence: Synthetic peptide
RANQSIASYLN

SEQ ID NO: 38 - protein, 7 aa, Artificial Sequence
  Description of Artificial Sequence: Synthetic peptide
GASSLQN

SEQ ID NO: 39 - protein, 9 aa, Artificial Sequence
  Description of Artificial Sequence: Synthetic peptide
QQSYSTEIT

SEQ ID NO: 40 - protein, 120 aa, Artificial Sequence
  Description of Artificial Sequence: Synthetic polypeptide
EVQVVESGGGLVQPGGSLRLSCAASGFTFRSYWMSWVRQAPGKGLEWVANIKQDGSERHYVDSVKGRFTISRDNAKTSLYLQMSSLRAEDTAVYYCAREGYFGSGYFDYWGQGTLVTVSS

SEQ ID NO: 41 - protein, 10 aa, Artificial Sequence
  Description of Artificial Sequence: Synthetic peptide
GFTFRSYWMS

SEQ ID NO: 42 - protein, 17 aa, Artificial Sequence
  Description of Artificial Sequence: Synthetic peptide
NIKQDGSERHYVDSVKG

SEQ ID NO: 43 - protein, 11 aa, Artificial Sequence
  Description of Artificial Sequence: Synthetic peptide
EGYFGSGYFDY

SEQ ID NO: 44 - protein, 107 aa, Artificial Sequence
  Description of Artificial Sequence: Synthetic polypeptide
DIQMTQSPSTLSASVGDRVIITCRASQSISRGLAWYQQKPGKAPKLLIYKASNLESGVPSRFSGSGSGTEFTLTISSLQPDDFAAYYCQQYSYYSHTFGQGTKLEIK

SEQ ID NO: 45 - protein, 11 aa, Artificial Sequence
  Description of Artificial Sequence: Synthetic peptide
RASQSISRGLA

SEQ ID NO: 46 - protein, 7 aa, Artificial Sequence
  Description of Artificial Sequence: Synthetic peptide
KASNLES

SEQ ID NO: 47 - protein, 9 aa, Artificial Sequence
  Description of Artificial Sequence: Synthetic peptide
QQYSYYSHT

SEQ ID NO: 48 - protein, 125 aa, Artificial Sequence
  Description of Artificial Sequence: Synthetic polypeptide
QGQVVESGGGVVQPGRSLRLSCAASGFTFSSYTLHWVRQAPGKGLEWVAVIWYDGSNKYYVDSVKGRFTISRDNSKNTLYLQMNSLRAEDTAVYYCAREYGSGSYYNVYYGMDVWGQGTTVTLSS

SEQ ID NO: 49 - protein, 10 aa, Artificial Sequence
  Description of Artificial Sequence: Synthetic peptide
GFTFSSYTLH

SEQ ID NO: 50 - protein, 17 aa, Artificial Sequence
  Description of Artificial Sequence: Synthetic peptide
VIWYDGSNKYYVDSVKG

SEQ ID NO: 51 - protein, 16 aa, Artificial Sequence
  Description of Artificial Sequence: Synthetic peptide
EYGSGSYYNVYYGMDV

SEQ ID NO: 52 - protein, 112 aa, Artificial Sequence
  Description of Artificial Sequence: Synthetic polypeptide
DIVMTQSPLSLPVTPGEPASISCRSSQSLLHSNGYNYLDWYLQKPGQSPHLLIYLASNRASGVPDRFSGSGSGTDFTLKISRVEAEDVGFYYCMQTLQIPLTFGGGTKVEIK

SEQ ID NO: 53 - protein, 16 aa, Artificial Sequence
  Description of Artificial Sequence: Synthetic peptide
RSSQSLLHSNGYNYLD

SEQ ID NO: 54 - protein, 7 aa, Artificial Sequence
  Description of Artificial Sequence: Synthetic peptide
LASNRAS

SEQ ID NO: 55 - protein, 9 aa, Artificial Sequence
  Description of Artificial Sequence: Synthetic peptide
MQTLQIPLT

SEQ ID NO: 56 - protein, 117 aa, Artificial Sequence
  Description of Artificial Sequence: Synthetic polypeptide
QVQLQESGPGLVKPSETLSLTCAVSGYSASGVYYWGWIRQPPGKGLEWIGNIYHSGSTYYNPSLERRVSISLDTSKNHFSLRLNFVTAADTAVYYCARDRFDAFDIWGQGTMVTVSS

SEQ ID NO: 57 - protein, 11 aa, Artificial Sequence
  Description of Artificial Sequence: Synthetic peptide
GYSASGVYYWG

SEQ ID NO: 58 - protein, 16 aa, Artificial Sequence
  Description of Artificial Sequence: Synthetic peptide
NIYHSGSTYYNPSLER

SEQ ID NO: 59 - protein, 8 aa, Artificial Sequence
  Description of Artificial Sequence: Synthetic peptide
DRFDAFDI

SEQ ID NO: 60 - protein, 107 aa, Artificial Sequence
  Description of Artificial Sequence: Synthetic polypeptide
EIVMTQSPATLSVSPGERATLSCRASQSINNILAWYQQKPGQAPRLLIYGASTRATGIPARFSGSGSGTEFTLTISSLQSEDFAVYYCQQYNNWPLTFGGGTKVEIK

SEQ ID NO: 61 - protein, 11 aa, Artificial Sequence
  Description of Artificial Sequence: Synthetic peptide
RASQSINNILA

SEQ ID NO: 62 - protein, 7 aa, Artificial Sequence
  Description of Artificial Sequence: Synthetic peptide
GASTRAT

SEQ ID NO: 63 - protein, 9 aa, Artificial Sequence
  Description of Artificial Sequence: Synthetic peptide
QQYNNWPLT

SEQ ID NO: 64 - protein, 121 aa, Artificial Sequence
  Description of Artificial Sequence: Synthetic polypeptide
QVQLVESGGGVVQPGRSLRLSCAASGFTFRSHGMHWVRQAPGKGLEWVAVIWYDGSSEYYADSVKGRFTISRDNSKNTLYLQMNSLRAEDTAVYYCARENVYGSGWFFDYWGQGTLVTVSS

SEQ ID NO: 65 - protein, 10 aa, Artificial Sequence
  Description of Artificial Sequence: Synthetic peptide
GFTFRSHGMH

SEQ ID NO: 66 - protein, 17 aa, Artificial Sequence
  Description of Artificial Sequence: Synthetic peptide
VIWYDGSSEYYADSVKG

SEQ ID NO: 67 - protein, 12 aa, Artificial Sequence
  Description of Artificial Sequence: Synthetic peptide
ENVYGSGWFFDY

SEQ ID NO: 68 - protein, 108 aa, Artificial Sequence
  Description of Artificial Sequence: Synthetic polypeptide
EIVMTQSPATLSVSPGERASLSCRASQSVGSNLAWYQQRPGQAPRLLIFGASTRATGIPARFSGSRSGTEFTLTISSLQSEDFALYYCQQYNNWPPWTFGQGTKLEIK

SEQ ID NO: 69 - protein, 11 aa, Artificial Sequence
  Description of Artificial Sequence: Synthetic peptide
RASQSVGSNLA

SEQ ID NO: 70 - protein, 10 aa, Artificial Sequence [sequence omitted]

SEQ ID NO: 71 - protein, 121 aa, Artificial Sequence
  Description of Artificial Sequence: Synthetic polypeptide
QVQLVESGGGVVQPGRSLRLSCAASGFTFRSHGMHWVRQAPGKGLEWVAVIWYDGSSDYYADSVKGRFTISRDNSKNTLFLQMNSLSAEDTAVYYCARENVYGSGWFFDYWGQGTLVTVSS

SEQ ID NO: 72 - protein, 17 aa, Artificial Sequence
  Description of Artificial Sequence: Synthetic peptide
VIWYDGSSDYYADSVKG

SEQ ID NO: 73 - protein, 108 aa, Artificial Sequence
  Description of Artificial Sequence: Synthetic polypeptide
EIVMTQSPATLSVSPGERASLSCRASQSVGSNLAWYQQKPGQAPRLLIFGASTRATGIPARFSGSRSGTEFTLTISSLQSEDFALYYCQQYNNWPPWTFGQGTKLEIK

SEQ ID NO: 74 - protein, 117 aa, Artificial Sequence
  Description of Artificial Sequence: Synthetic polypeptide
EVQLLESGGGLVQPGGSLRLSCAASGFTFSNYAMTWVRQAPGKGLEWVSSISISRAGTYYADSVKGRFTISRDNSKNTLNLQMNSLRAEDTAEYYCAREYYYGMDVWGQGTTVTVSS

SEQ ID NO: 75 - protein, 10 aa, Artificial Sequence
  Description of Artificial Sequence: Synthetic peptide
GFTFSNYAMT

SEQ ID NO: 76 - protein, 17 aa, Artificial Sequence
  Description of Artificial Sequence: Synthetic peptide
SISISRAGTYYADSVKG

SEQ ID NO: 77 - protein, 8 aa, Artificial Sequence
  Description of Artificial Sequence: Synthetic peptide
EYYYGMDV

SEQ ID NO: 78 - protein, 107 aa, Artificial Sequence
  Description of Artificial Sequence: Synthetic polypeptide
EIVLTQSPATLSLSPGERATLSCRASQSVSSYLAWYQQKPGQTPRLLIYDASNRATGIPARFSGSGSGTDFTLTISSLETEDFAVYYCQQLINWPLTFGGGTKLEIK

SEQ ID NO: 79 - protein, 11 aa, Artificial Sequence
  Description of Artificial Sequence: Synthetic peptide
RASQSVSSYLA

SEQ ID NO: 80 - protein, 7 aa, Artificial Sequence
  Description of Artificial Sequence: Synthetic peptide
DASNRAT

SEQ ID NO: 81 - protein, 9 aa, Artificial Sequence
  Description of Artificial Sequence: Synthetic peptide
QQLINWPLT

SEQ ID NO: 82 - protein, 107 aa, Artificial Sequence
  Description of Artificial Sequence: Synthetic polypeptide
DIQMTQSPSSLSASVGDRVIITCRASQGISNYLAWFQQKPGKAPNLLIYAASTLRSGVPSRFSGSGSGTDFTLTISSLQPEDVATYYCQKYNSAPYTFGQGTKVEIK

SEQ ID NO: 83 - protein, 117 aa, Artificial Sequence
  Description of Artificial Sequence: Synthetic polypeptide
EVQLLESGADLVQPGGSLRLSCAASGFTFSSYAMSWVRQAPGKGLEWVSTIRISGGTTYYADSVKGRFTISRDNSKNTLYLQMNSLRAEDTAVYYCVRDYYNGMDVWGQGTTVTVSS

SEQ ID NO: 84 - protein, 10 aa, Artificial Sequence
  Description of Artificial Sequence: Synthetic peptide
GFTFSSYAMS

SEQ ID NO: 85 - protein, 17 aa, Artificial Sequence
  Description of Artificial Sequence: Synthetic peptide
TIRISGGTTYYADSVKG

SEQ ID NO: 86 - protein, 8 aa, Artificial Sequence
  Description of Artificial Sequence: Synthetic peptide
DYYNGMDV

SEQ ID NO: 87 - protein, 107 aa, Artificial Sequence
  Description of Artificial Sequence: Synthetic polypeptide
EIVLTQSPATLSLSPGERATLSCRASQRVSSYLAWYQQKPGQAPRLLIYDASNRATGIPARFSGSGSGTDFTLTISSLEPEDFAVYYCQQRSYWPPAFGQGTKLEIK

SEQ ID NO: 88 - protein, 11 aa, Artificial Sequence
  Description of Artificial Sequence: Synthetic peptide
RASQRVSSYLA

SEQ ID NO: 89 - protein, 9 aa, Artificial Sequence
  Description of Artificial Sequence: Synthetic peptide
QQRSYWPPA

SEQ ID NO: 90 - protein, 117 aa, Artificial Sequence
  Description of Artificial Sequence: Synthetic polypeptide
EVQLLESGGGLVQRGGSLRLSCAASGFTFSSYAMSWVRQAPGKGLEWVSSISGSGDSTNYADSVKGRFTISRDNSKNTLHLQMNSLRAEDTAVYYCVRDYYYGMDVWGHGTTVTVSS

SEQ ID NO: 91 - protein, 17 aa, Artificial Sequence
  Description of Artificial Sequence: Synthetic peptide
SISGSGDSTNYADSVKG

SEQ ID NO: 92 - protein, 8 aa, Artificial Sequence
  Description of Artificial Sequence: Synthetic peptide
DYYYGMDV

SEQ ID NO: 93 - protein, 107 aa, Artificial Sequence
  Description of Artificial Sequence: Synthetic polypeptide
EIVLTQSPATLSLSPGERATLSCRASQSVNSYLAWYQQKPGQAPRLLIYDASNRATGIPARFSGSGSGTDFTLTISSLEPEDFAVYYCQQRSYWPITFGQGTRLEIK

SEQ ID NO: 94 - protein, 11 aa, Artificial Sequence
  Description of Artificial Sequence: Synthetic peptide
RASQSVNSYLA

SEQ ID NO: 95 - protein, 9 aa, Artificial Sequence
  Description of Artificial Sequence: Synthetic peptide
QQRSYWPIT

SEQ ID NO: 96 - protein, 117 aa, Artificial Sequence
  Description of Artificial Sequence: Synthetic polypeptide
EAQLLESGGGLVQPGGSLRLSCAASGFTFSSYAMSWVRQAPGKGLEWVSTISGSGGSTHYADSVKGRFTISRDNSKNTLYLQMNSLRAEDTAVYYCVRDYYYGMDVWGQGTTVTVSS

SEQ ID NO: 97 - protein, 17 aa, Artificial Sequence
  Description of Artificial Sequence: Synthetic peptide
TISGSGGSTHYADSVKG

SEQ ID NO: 98 - protein, 107 aa, Artificial Sequence
  Description of Artificial Sequence: Synthetic polypeptide
EIVLTQSPATLSLSPGERATLSCRASQSVSSYLAWYQQKPGQAPRLLIYDASNRATGIPARFSGSGSGTDFTLTISSLEPEDFAVYYCQQRSYWPPTFGQGTKLEIK

SEQ ID NO: 99 - protein, 9 aa, Artificial Sequence
  Description of Artificial Sequence: Synthetic peptide
QQRSYWPPT

SEQ ID NO: 100 - protein, 121 aa, Artificial Sequence
  Description of Artificial Sequence: Synthetic polypeptide
QVQLVESGGGVVQPGRSLRLSCAASGFTFSSYGMHWVRQAPGKGLEWVAVIWYDGSKKYYVDSVQGRFTISRDNSKNTLYLQMNSLRGEDTAVYYCARDGGAVADNWIDSWGQGTLVTVSS

SEQ ID NO: 101 - protein, 10 aa, Artificial Sequence
  Description of Artificial Sequence: Synthetic peptide
GFTFSSYGMH

SEQ ID NO: 102 - protein, 17 aa, Artificial Sequence
  Description of Artificial Sequence: Synthetic peptide
VIWYDGSKKYYVDSVQG

SEQ ID NO: 103 - protein, 107 aa, Artificial Sequence
  Description of Artificial Sequence: Synthetic polypeptide
DIQMTQSPSSLSASVGDRVTLTCRASQNIRSYLNWYQQKPGKAPKLLIFAASSLPSGVPSRFSGSGSVTDFTLTVSSLQPEDFATYSCQQSYSTPYTFGQGTKLEIK

SEQ ID NO: 104 - protein, 11 aa, Artificial Sequence
  Description of Artificial Sequence: Synthetic peptide
RASQNIRSYLN

SEQ ID NO: 105 - protein, 7 aa, Artificial Sequence
  Description of Artificial Sequence: Synthetic peptide
AASSLPS

SEQ ID NO: 106 - protein, 117 aa, Artificial Sequence
  Description of Artificial Sequence: Synthetic polypeptide
EEQLLESGADLAQPGGSLRLSCAASGFTFSSYAMSWVRQAPGKGLEWVSTIRISGDTTYYADSVKGRFTISRDNSKNTLFLQMNSLRAEDTAVYYCVRDYYNGMDVWGHGTTVTVSS

SEQ ID NO: 107 - protein, 17 aa, Artificial Sequence
  Description of Artificial Sequence: Synthetic peptide
TIRISGDTTYYADSVKG

SEQ ID NO: 108 - protein, 107 aa, Artificial Sequence; identical to SEQ ID NO: 87
  Description of Artificial Sequence: Synthetic polypeptide

SEQ ID NO: 109 - protein, 121 aa, Artificial Sequence
  Description of Artificial Sequence: Synthetic polypeptide
QVQLVQSGAEVKKPGASVKVSCKASGYTFTGYYMHWVRQAPGQGLEWMGWINPNSGGTNYAQKFQGRVTMTRDTSISTAYMELSRLRSDDTAVYYCAREAVAGTSDAFDIWGQGTMVTVSS

SEQ ID NO: 110 - protein, 10 aa, Artificial Sequence
  Description of Artificial Sequence: Synthetic peptide
GYTFTGYYMH

SEQ ID NO: 111 - protein, 17 aa, Artificial Sequence
  Description of Artificial Sequence: Synthetic peptide
WINPNSGGTNYAQKFQG

SEQ ID NO: 112 - protein, 12 aa, Artificial Sequence
  Description of Artificial Sequence: Synthetic peptide
EAVAGTSDAFDI

SEQ ID NO: 113 - protein, 107 aa, Artificial Sequence
  Description of Artificial Sequence: Synthetic polypeptide
DIQMTQSPSSLSASVGDRVTITCRANQSIASYLNWYQQKPGKVPKLLIYGASSLQNGVPSRFSGSGSRTDFTLTISSLQPEDFATYYCQQSYSTEITFGQGTRLEIK

SEQ ID NO: 114 - protein, 107 aa, Artificial Sequence
  Description of Artificial Sequence: Synthetic polypeptide
DIQMTQSPSSLSASVGDRVAITCRASQSIASYLNWYQQKPGKAPKLLIYGASSLQNGVPSRFSGSGSRTDFTLTISSLQPEDFATYYCQQSYSTEITFGQGTRLEIK

SEQ ID NO: 115 - protein, 11 aa, Artificial Sequence
  Description of Artificial Sequence: Synthetic peptide
RASQSIASYLN

SEQ ID NO: 116 - protein, 120 aa, Artificial Sequence
  Description of Artificial Sequence: Synthetic polypeptide
QVQLVESGGGVVQPGRSLRLSCAASGFTFRNYGMHWVRQAPGKGLEWVAVIWYDGSNKFYADSVKGRFTISRDNSKNTLYLQMNSLRVEDTAVYYCAREEGIAVAPFDYWGQGTLVTVSS

SEQ ID NO: 117 - protein, 10 aa, Artificial Sequence
  Description of Artificial Sequence: Synthetic peptide
GFTFRNYGMH

SEQ ID NO: 118 - protein, 121 aa, Artificial Sequence
  Description of Artificial Sequence: Synthetic polypeptide
QVQLVESGGGMVQPGRSLRLSCTASGFTFSSHGMHWVRQAPGKGLEWVAVIWFDGSNEYYVDSVKGRFTISRDNSKNTLYLQMNSLRAEDTAVYYCARENVYGSGWFFDYWGQGTLVTVSS

SEQ ID NO: 119 - protein, 17 aa, Artificial Sequence
  Description of Artificial Sequence: Synthetic peptide
VIWFDGSNEYYVDSVKG

SEQ ID NO: 120 - protein, 108 aa, Artificial Sequence
  Description of Artificial Sequence: Synthetic polypeptide
EIVMTQSPATLSVSPGERASLSCRASQSVGSNLAWYQQKPGQAPRLLIFGASTRATGIPARFSGSRSGTEFTLTISSLQSEDFALYYCQQYNNWPPWTFGQGTKVEIK

SEQ ID NO: 121 - protein, 121 aa, Artificial Sequence
  Description of Artificial Sequence: Synthetic polypeptide
QLQLVESGGGVVQPGRSLRLSCAASGFTFSSYGMHWVRQAPGKGLEWVAVIWYDGSSEYYADSVKGRFTISRDNSKNTLYLQMNSLRAEDTAVYYCARENVYGSGWFFDYWGQGTLVTVSS

SEQ ID NO: 122 - protein, 108 aa, Artificial Sequence; identical to SEQ ID NO: 120
  Description of Artificial Sequence: Synthetic polypeptide

SEQ ID NO: 123 - protein, 121 aa, Artificial Sequence
  Description of Artificial Sequence: Synthetic polypeptide
QLQLVESGGGVVQPGRSLRLSCAASGFTFSSHGMHWVRQAPGKGLEWVAVIWYDGSSEYYADSVKGRFTISRDNSKNTLYLQMNSLRAEDTAVYYCARENVYGSGWFFDYWGQGSLVTVSS

SEQ ID NO: 124 - protein, 108 aa, Artificial Sequence; identical to SEQ ID NO: 73
  Description of Artificial Sequence: Synthetic polypeptide

SEQ ID NO: 125 - protein, 121 aa, Artificial Sequence
  Description of Artificial Sequence: Synthetic polypeptide
QLQLVESGGGVVQFGRSLRLSCAASGFTFSSHGMHWVRQAPGKGLEWVAVIWYDGSSEYYADSVKGRFTISRDNSKNTLYLQMNSLRAEDTAVYYCARENVYGSGWFFDYWGQGTLVTVSS

SEQ ID NO: 126 - protein, 108 aa, Artificial Sequence; identical to SEQ ID NO: 73
  Description of Artificial Sequence: Synthetic polypeptide

SEQ ID NO: 127 - protein, 121 aa, Artificial Sequence
  Description of Artificial Sequence: Synthetic polypeptide
QLQLVESGGGVVQPGRSLRLSCAASGFTFSSYGMHWVRQAPGKGLEWVAVIWYDGSSEYYADSVKGRFTISRDNSKNTLFLQMNSLRADDTAVYYCARENVYGSGWFFDYWGQGTLVTVSS

SEQ ID NO: 128 - protein, 108 aa, Artificial Sequence
  Description of Artificial Sequence: Synthetic polypeptide
EIVMTQSPATLSVSPGERASLSCRASQSVGSNLAWYQQKPGQAPRLLIFGASTRATGIPARFSGSRSGTEFTLTISSLQSEDFALYYCQQYDNWPPWTFGQGTKLEIK

SEQ ID NO: 129 - protein, 10 aa, Artificial Sequence
  Description of Artificial Sequence: Synthetic peptide
QQYDNWPPWT

SEQ ID NO: 130 - protein, 121 aa, Artificial Sequence
  Description of Artificial Sequence: Synthetic polypeptide
QVQLVESGGGVVQPGRSLRLSCAASGFTLSGYGMHWVRQAPGKGLEWVAVIWYDGSNKYYADSVKGRFTISRDNSKNMLFLQMNSLRAEDTAVYYCVRENGFGSGWFFDYWGQGNLVTVSS

SEQ ID NO: 131 - protein, 10 aa, Artificial Sequence
  Description of Artificial Sequence: Synthetic peptide
GFTLSGYGMH

SEQ ID NO: 132 - protein, 17 aa, Artificial Sequence
  Description of Artificial Sequence: Synthetic peptide
VIWYDGSNKYYADSVKG

SEQ ID NO: 133 - protein, 12 aa, Artificial Sequence
  Description of Artificial Sequence: Synthetic peptide
ENGFGSGWFFDY

SEQ ID NO: 134 - protein, 108 aa, Artificial Sequence
  Description of Artificial Sequence: Synthetic polypeptide
EIVMTQSPATLSVSPGERATLSCRTSQSVSRDLAWYQQKPGQAPRLLIYGASTRATGIPVRFSGSGSGTEFTLTISSLQSEDFAVYYCQQYNNWPPWTFGQGTKLEIK

SEQ ID NO: 135 - protein, 11 aa, Artificial Sequence
  Description of Artificial Sequence: Synthetic peptide
RTSQSVSRDLA

SEQ ID NO: 136 - protein, 125 aa, Artificial Sequence
  Description of Artificial Sequence: Synthetic polypeptide
QGQLVESGGGVVQPGRSLRLSCAASGFTFSSYTLHWVRQAPGKGLEWVAVIWYDGSNKYYVDSVKGRFTISRDNSKNTLYLQMNSLRAEDTAVYYCAREYGSGSYYNVYYGMDVWGQGTTVTVSS

SEQ ID NO: 137 - protein, 112 aa, Artificial Sequence
  Description of Artificial Sequence: Synthetic polypeptide
DIVMTQSPLSLPVTPGEPASISCRSSQSLLHSNGYKYLDWYLQKAGQSPHLLIYLGSNRASGVPDRFSGSGSGTDFTLKISRVEAEDVGFYYCMQTLQIPLTFGGGTKLEIK

SEQ ID NO: 138 - protein, 16 aa, Artificial Sequence
  Description of Artificial Sequence: Synthetic peptide
RSSQSLLHSNGYKYLD

SEQ ID NO: 139 - protein, 7 aa, Artificial Sequence
  Description of Artificial Sequence: Synthetic peptide
LGSNRAS

SEQ ID NO: 140 - protein, 120 aa, Artificial Sequence
  Description of Artificial Sequence: Synthetic polypeptide
EVQVVESGGGLVQPGGSLRLSCATSGFTFRSYWMTWVRQAPGKGLEWVANIKQDGSERHYVDSVKGRFTISRDNAKTSLYLQMSSLRAEDTAMYYCAREGYYGSGYFDYWGQGTLVTVSS

SEQ ID NO: 141 - protein, 10 aa, Artificial Sequence
  Description of Artificial Sequence: Synthetic peptide
GFTFRSYWMT

SEQ ID NO: 142 - protein, 11 aa, Artificial Sequence
  Description of Artificial Sequence: Synthetic peptide
EGYYGSGYFDY

SEQ ID NO: 143 - protein, 107 aa, Artificial Sequence
  Description of Artificial Sequence: Synthetic polypeptide
DIQMTQSPSTLSASVGDRVIITCRASQSISRGLAWYQQKPGKAPKLLIYKASNLESGVPSRFSGSGSGTEFTLTISSLQPDDFAAYYCQQYSYYSHTFGQGTKVEIK

SEQ ID NO: 144 - protein, 120 aa, Artificial Sequence
  Description of Artificial Sequence: Synthetic polypeptide
EVQLVESGGGLVQPGGSLRLSCAASGFTLSFYWMTWVRQAPGKGLEWVANIKQDGNEKNYVDSVKGRFTISKDNAKKSVFLQMNSLRAEDTAVYYCAREGYFGSGYFDYWGQGTLVTVSS

SEQ ID NO: 145 - protein, 10 aa, Artificial Sequence
  Description of Artificial Sequence: Synthetic peptide
GFTLSFYWMT

SEQ ID NO: 146 - protein, 17 aa, Artificial Sequence
  Description of Artificial Sequence: Synthetic peptide
NIKQDGNEKNYVDSVKG

SEQ ID NO: 147 - protein, 107 aa, Artificial Sequence
  Description of Artificial Sequence: Synthetic polypeptide
DIQMTQSPSTLSASVGDRVTITCRASQSINSWLAWYQQKPGKAPKLLIYKASTLESGVPSRFSGSGSGTEFTLTISSLQPDDFAPYYCQHYNSYPHTFGQGTKVEIK

SEQ ID NO: 148 - protein, 11 aa, Artificial Sequence
  Description of Artificial Sequence: Synthetic peptide
RASQSINSWLA

SEQ ID NO: 149 - protein, 7 aa, Artificial Sequence
  Description of Artificial Sequence: Synthetic peptide
KASTLES

SEQ ID NO: 150 - protein, 9 aa, Artificial Sequence
  Description of Artificial Sequence: Synthetic peptide
QHYNSYPHT

SEQ ID NO: 151 - protein, 120 aa, Artificial Sequence
  Description of Artificial Sequence: Synthetic polypeptide
EVQLVESGGGLVQPGGSLRLSCAASGFTFSSYWMSWVRQAPGKGLEWVANIKQDGSEKHYVDSVKGRFTISRDNAKNSLYLQMNSLRAEDTAVYYCAREGYFGSGYFDYWGQGTLVTVSS

SEQ ID NO: 152 - protein, 10 aa, Artificial Sequence
  Description of Artificial Sequence: Synthetic peptide
GFTFSSYWMS

SEQ ID NO: 153 - protein, 17 aa, Artificial Sequence
  Description of Artificial Sequence: Synthetic peptide
NIKQDGSEKHYVDSVKG

SEQ ID NO: 154 - protein, 107 aa, Artificial Sequence
  Description of Artificial Sequence: Synthetic polypeptide
DIQLTQSPSFLSASVGDRVTITCRASQGISSYLAWYQQKPGKAPKLLIYAASTLQSGVPSRFSGSGSGTEFTLTISSLQPEDFATYYCQQYSFYSHTFGQGTKLEIK

SEQ ID NO: 155 - protein, 11 aa, Artificial Sequence
  Description of Artificial Sequence: Synthetic peptide
RASQGISSYLA

SEQ ID NO: 156 - protein, 7 aa, Artificial Sequence
  Description of Artificial Sequence: Synthetic peptide
AASTLQS

SEQ ID NO: 157 - protein, 9 aa, Artificial Sequence
  Description of Artificial Sequence: Synthetic peptide
QQYSFYSHT

SEQ ID NO: 158 - protein, 120 aa, Artificial Sequence
  Description of Artificial Sequence: Synthetic polypeptide
EVQLVESGGGLVQPGGSLRLSCAASGFTLSFYWMTWVRQAPGKGLEWVANIKQDGNEKNFVDSVKGRFTISRDNAKKSVFLQMNSLRAEDTAVYYCAREGYFGSGYFDYWGQGTLVTVSS

SEQ ID NO: 159 - protein, 17 aa, Artificial Sequence
  Description of Artificial Sequence: Synthetic peptide
NIKQDGNEKNFVDSVKG

SEQ ID NO: 160 - protein, 107 aa, Artificial Sequence
  Description of Artificial Sequence: Synthetic polypeptide
DIQMTQSPSTLSASVGDRVTITCRASQSINSWLAWYQQKPGKAPKLLIYKASSLESGVPSRFSGSGSGTEFTLTISSLQPDDFATYYCQQYNSYPHTFGQGTKLEIK

SEQ ID NO: 161 - protein, 7 aa, Artificial Sequence
  Description of Artificial Sequence: Synthetic peptide
KASSLES

SEQ ID NO: 162 - protein, 9 aa, Artificial Sequence
  Description of Artificial Sequence: Synthetic peptide
QQYNSYPHT

SEQ ID NO: 163 - protein, 119 aa, Artificial Sequence
  Description of Artificial Sequence: Synthetic polypeptide
QVQLQESGPGLVKPLGTLSLTCAVSGGSISNSNWWSWVRQPPGKGLEWIGEIYHSGSTNYNPSLKSRVTIALDWSKNQFSLQLRSVTAADTAVYYCARYGSGPFGGDCWGQGTLVTVSS

SEQ ID NO: 164 - protein, 11 aa, Artificial Sequence
  Description of Artificial Sequence: Synthetic peptide
GGSISNSNWWS

SEQ ID NO: 165 - protein, 16 aa, Artificial Sequence
  Description of Artificial Sequence: Synthetic peptide
EIYHSGSTNYNPSLKS

SEQ ID NO: 166 - protein, 10 aa, Artificial Sequence
  Description of Artificial Sequence: Synthetic peptide
YGSGPFGGDC

SEQ ID NO: 167 - protein, 107 aa, Artificial Sequence
  Description of Artificial Sequence: Synthetic polypeptide
DIQLTQSPSFLSASVGDRVTISCRASQGISSYLAWYQQKPGKAPKLLIYAASTLQGGVPSRFSGSGSGTTFTLTISSLQPEDFATYYCQQLNTYPFTFGPGTKLEIK

SEQ ID NO: 168 - protein, 7 aa, Artificial Sequence
  Description of Artificial Sequence: Synthetic peptide
AASTLQG

SEQ ID NO: 169 - protein, 9 aa, Artificial Sequence
  Description of Artificial Sequence: Synthetic peptide
QQLNTYPFT

SEQ ID NO: 170 - protein, 119 aa, Artificial Sequence
  Description of Artificial Sequence: Synthetic polypeptide
QVQLQESGPGLVKPLGTLSLTCAVSGGSISNSNWWSWVRQPPGKGLEWIGEIYHSGSTNYNPSLKSRVTIALDWSKNQFSLQLRSVTAADTAVYYCARYGSGPFGGDYWGQGTLVTVSS

SEQ ID NO: 171 - protein, 10 aa, Artificial Sequence
  Description of Artificial Sequence: Synthetic peptide
YGSGPFGGDY

SEQ ID NO: 172 - protein, 107 aa, Artificial Sequence; identical to SEQ ID NO: 167
  Description of Artificial Sequence: Synthetic polypeptide

SEQ ID NO: 173 - protein, 123 aa, Artificial Sequence
  Description of Artificial Sequence: Synthetic polypeptide
QVQIKESGPGLVKPSETLSLTCAVSGFSFSSGYYWGWIRQPPGKGLEWLGSFFHNGNTYYNPSLRSRVTISVDTSKNHFSLKLTSVTAADTAVYYCAGFGDLPHYHYYVMDVWGQGTTVTVSS

SEQ ID NO: 174 - protein, 11 aa, Artificial Sequence
  Description of Artificial Sequence: Synthetic peptide
GFSFSSGYYWG

SEQ ID NO: 175 - protein, 16 aa, Artificial Sequence
  Description of Artificial Sequence: Synthetic peptide
SFFHNGNTYYNPSLRS

SEQ ID NO: 176 - protein, 14 aa, Artificial Sequence
  Description of Artificial Sequence: Synthetic peptide
FGDLPHYHYYVMDV

SEQ ID NO: 177 - protein, 108 aa, Artificial Sequence
  Description of Artificial Sequence: Synthetic polypeptide
EIVLTQSPATLSLSPGERATLSCRASQSVSSYLAWYQQKPGQAPRLLIYDASNRAIGIPARFSGSGSGTDFTLTISSLEPEDFAVYYCQQRSNWPPYTFGQGTKLEIK

SEQ ID NO: 178 - protein, 7 aa, Artificial Sequence
  Description of Artificial Sequence: Synthetic peptide
DASNRAI

SEQ ID NO: 179 - protein, 10 aa, Artificial Sequence
  Description of Artificial Sequence: Synthetic peptide
QQRSNWPPYT

SEQ ID NO: 180 - protein, 123 aa, Artificial Sequence
  Description of Artificial Sequence: Synthetic polypeptide
QVQPKESGPGVVKPSETLSLTCAVSGFPISRGYYWGWIRQPPGKGLEWIGNIFHSGTTYYNPSLKSRVTISVDTSKNQISLKLTSVTAADTAVYYCVGFGDLPHYQYYVMDIWGQGTTVTVSS

SEQ ID NO: 181 - protein, 11 aa, Artificial Sequence
  Description of Artificial Sequence: Synthetic peptide
GFPISRGYYWG

SEQ ID NO: 182 - protein, 16 aa, Artificial Sequence
  Description of Artificial Sequence: Synthetic peptide
NIFHSGTTYYNPSLKS

SEQ ID NO: 183 - protein, 14 aa, Artificial Sequence
  Description of Artificial Sequence: Synthetic peptide
FGDLPHYQYYVMDI

SEQ ID NO: 184 - protein, 108 aa, Artificial Sequence
  Description of Artificial Sequence: Synthetic polypeptide
EIVLTQSPATLSLSPGERATLSCRASQSVSSYLAWYQQKPGQAPRLLIYDASNRATGIPARFSGSGSGTDFTLTISSLEPEDFAVYYCQQRSNWPPYTFGQGTKLEIK

SEQ ID NO: 185 - protein, 117 aa, Artificial Sequence
  Description of Artificial Sequence: Synthetic polypeptide
QVQLQESGPGLVKPSETLSLTCAVSGYSASGLYYWAWIRQPPGKGLEWIGNIYHSGRTYYNPSLESRVSISLDTSKHQVSLKLKSVTYADTAVYFCARDRFDGFDIWGQGTMVTVSS

SEQ ID NO: 186 - protein, 11 aa, Artificial Sequence
  Description of Artificial Sequence: Synthetic peptide
GYSASGLYYWA

SEQ ID NO: 187 - protein, 16 aa, Artificial Sequence
  Description of Artificial Sequence: Synthetic peptide
NIYHSGRTYYNPSLES

SEQ ID NO: 188 - protein, 8 aa, Artificial Sequence
  Description of Artificial Sequence: Synthetic peptide
DRFDGFDI

SEQ ID NO: 189 - protein, 107 aa, Artificial Sequence
  Description of Artificial Sequence: Synthetic polypeptide
EIVMTQSPATLSVSPGERATLSCRASQTINNILAWYQQKPGQAPRLLIYGASTRATGIPARFSGSGSGTEFTLTISSLQSEDFAVYYCQQYNNWPLTFGGGTKLEIK

SEQ ID NO: 190 - protein, 11 aa, Artificial Sequence
  Description of Artificial Sequence: Synthetic peptide
RASQTINNILA

SEQ ID NO: 191 - DNA, 342 bp, Artificial Sequence
  Description of Artificial Sequence: Synthetic polynucleotide
caggtggagctgcaggagtcgggcccaggactggtgaagccttcggacaccctgtccctcacctgcactgtcactggtggctccatcagtacttactactggagctggatccggcagcccccagggaagggactggagtggattgggtatatcttttacactgggaccaccaactacaacccctccctcaagagtcgagtcaccatatcagtagacgcgtccaagaaccagttctccctgaagttgaactctgtgaccgctgcggacacggccgtgtattactgtgcgagagatgggagcctggactactggggccagggagccctggtcaccgtctcctca

SEQ ID NO: 192 - DNA, 321 bp, Artificial Sequence
  Description of Artificial Sequence: Synthetic polynucleotide
gacatccagatgacccagtctccatcctccctgtctgcatctgtaggagacagagtcaccatcacttgccgggcaagtcagagcattagcaactatttaaattggtatcagcagaaaccagggaaagcccctaagctcctgatctttgttgcatcccttttgcaaagtggggtcccatcaaggttcagtggcagtggatctgggacagatttcactctcaccatcagcagtctgcaacctgaagattttgcaacttactactgtcaacagagttacagtaccccattcactttcggccctgggaccaagctggagatcaaa

SEQ ID NO: 193 - DNA, 372 bp, Artificial Sequence
  Description of Artificial Sequence: Synthetic polynucleotide
caggtgcagctggtggagtctgggggaggcgtggtccagcctgggaggtccctgagaatctcctgtgcagcgtctggattcaccttcaggagctatggcatgcactgggtccgccaggctccaggcaagggactggagtgggtggcaattatctggcatgatgaaagttataaatattatgtagactccgtgaagggccgattcaccatctccagagacaattccaagaacacgctgtatctgcaaatgaacagcctgagagccgaggacacggctgtgtattattgtgcgagaggcgattactatggttcggggagttattatgatgcttttgatatctggggccaagggacaatggtcaccgtctcctca

SEQ ID NO: 194 - DNA, 321 bp, Artificial Sequence
  Description of Artificial Sequence: Synthetic polynucleotide
gacatccagatgacccagtctccatcctccctgtctgcatctgtaggagacagagtcatcatcacttgccgggcgagtcaaggcattagcaattatttagcctggtttcagcagaaaccagggaaatgtcctaacctcctgatctatgctgcatccactttgcgatcaggggtcccatctcggttcagtggcagtggatctgggacagatttcactctcaccatcagcagcctgcagcctgaagatgttgcaacttattactgtcaaaagtataacagtgccccgtacacttttggccaggggaccaaggtggagatcaaa

SEQ ID NO: 195 - DNA, 363 bp, Artificial Sequence
  Description of Artificial Sequence: Synthetic polynucleotide
caggtgcagctggtggagtctgggggaggcgtggtccagcctgggaggtccctgagactctcctgtgcagcgtctggattcaccttcagtcactatggcatgcactgggtccgccaggctccaggcaaggggctggagtgggtggcagttatatggtatgatggaagtaaaaaatactatgtagactccgtgaagggccgattcaccatctccagagacaattccaagaacacgctgtatctgcaaatgaacagcctgagaggcgaggacacggctgtgtattactgtgcgagagatgggggagcagtggctgacaactggatcgactcctggggccagggaaccctggtcaccgtctcctca

SEQ ID NO: 196 - DNA, 321 bp, Artificial Sequence
  Description of Artificial Sequence: Synthetic polynucleotide
gacatccagatgacccagtctccatcctccctgtctgcatctgtaggagacagagtcactatcacttgccgggcaagtcagagcattagaagctatttaaattggtatcagcagaaacccgggaaagcccctaagctcctgatctttgctgcatccagtttgcaaagtggggtcccatccaggttcagtggcagtggatctgggacagatttcactctcaccgtcagcagtctgcaacctgaagattttgcaacttactcctgtcaacaaagttacagtaccccgtacacttttggccaggggaccaaggtggagatcaaa

SEQ ID NO: 197 - DNA, 360 bp, Artificial Sequence
  Description of Artificial Sequence: Synthetic polynucleotide
caggtgcagttggtggagtctgggggaggcgtggtccagcctggggggtccctgagactctcctgtgcagcgtctggattcaccttcagtagccatggcatgcactgggtccgccaggctccaggcaaggggctggagtgggtggcagttatatggtatgatggaagtaataaattctatacagactccgtgcagggccgattcaccatttccagagacaattccaagaacacgctgaatctgcaaatgaacagtctgagagccgaggacacggctgtatattactgtgcgagagagggtttgagggccgggtactactttgacttctggggccagggaaccctggtcaccgtctcctca

SEQ ID NO: 198 - DNA, 321 bp, Artificial Sequence
  Description of Artificial Sequence: Synthetic polynucleotide
gacatccagatgacccagtctccatcctccctgtctgcatctgtaggagacagagtcaccatcacttgccgggcaagtcagaggattagcttctattcaaattggtatcagcagaaaccagggaaagcccctaagctcctgatctatgctgcatccagtttgcaaagtggggtcccatcaaggttcagtggcagtggctctgggacagatttcactctcaccatcagcagtctgcaacctgaagattttgcaacttacttctgtcaacagagtcacagtaccccgctcactttcggcggagggaccaagctggagatcaaa

SEQ ID NO: 199 - DNA, 360 bp, Artificial Sequence
  Description of Artificial Sequence: Synthetic polynucleotide
caggtgcagctggtggagtctgggggaggcgtggtccagcctgggaggtccctgcgactctcctgtgcagcgtctggattcaccttcaggaactatggcattcactgggtccgccaggctccaggcaaggggctggagtgggtggcagttatatggtatgatggaagtaataaattctatgcagactccgtgaagggccgattcaccatctccagagacaattccaagaacacgctgtatctgcaaatgaacagcctgagagtcgaggacacggctgtatattactgtgcgagagaggaggggatagcagtggccccctttgactactggggccagggaaccctggtcaccgtctcctca

SEQ ID NO: 200 - DNA, 321 bp, Artificial Sequence
  Description of Artificial Sequence: Synthetic polynucleotide
gacatccagatgacccagtctccatcctccctgtctgcatctgtaggagacagagtcgccatcacttgccgggcaaatcagagtattgccagttatttaaattggtatcagcagaaaccagggaaagcccctaaactcctgatctatggtgcatccagtttgcaaaatggggtcccatcaaggttcagtggcagtggatctaggacagatttcactctcaccatcagcagtctgcaacctgaagattttgcaacttactactgtcaacagagttacagcaccgagatcaccttcggccaagggacacgactggagattaaa

SEQ ID NO: 201 - DNA, 360 bp, Artificial Sequence
  Description of Artificial Sequence: Synthetic polynucleotide
gaggtgcaggtggtggagtctgggggaggcttggtccagcctggggggtccctgagactctcctgtgcagcctctggattcacctttagaagctattggatgagctgggtccgccaggctccagggaaggggctggagtgggtggccaacataaagcaggatggaagtgagagacactatgtggactctgtgaagggccgattcaccatctccagagacaacgccaagacatcactgtatctgcaaatgagcagcctgagagccgaggacacggctgtgtattactgtgcgagagaggggtactttggttcgggctactttgactactggggccagggaaccctggtcaccgtctcctca

SEQ ID NO: 202 - DNA, 321 bp, Artificial Sequence
  Description of Artificial Sequence: Synthetic polynucleotide
gacatccagatgacccagtctccctccaccctgtctgcatctgtaggagacagagtcatcatcacttgccgggccagtcagagtattagtagggggttggcctggtatcagcagaaaccagggaaagcccctaaactcttgatctataaggcgtctaatttagaaagtggggtcccatcaaggttcagcggcagtggatctgggacagaattcactctcaccatcagcagcctgcagcctgatgattttgcagcttattactgccaacagtatagttattattctcacacttttggccaggggaccaagctggagatcaaa

SEQ ID NO: 203 - DNA, 375 bp, Artificial Sequence
  Description of Artificial Sequence: Synthetic polynucleotide
caggggcaggtggtggagtctgggggaggcgtggtccagcctgggaggtccctgagactctcctgtgcagcgtctggattcaccttcagtagttataccttgcactgggtccgccaggctccaggcaaggggctggagtgggtggcagtcatatggtatgatggaagtaataagtattatgtagactccgtgaagggccgattcaccatctccagagacaattccaagaacacgctgtatctgcaaatgaacagcctgagagccgaggacacggctgtgtattactgtgcgagagagtatggttcggggagttattataacgtctactacggtatggacgtctggggccaggggaccacggtcaccctctcctca

SEQ ID NO: 204 - DNA, 336 bp, Artificial Sequence
  Description of Artificial Sequence: Synthetic polynucleotide
gatattgtgatgactcagtctccactctccctgcccgtcacccctggagagccggcctccatctcctgcaggtctagtcagagcctccttcatagtaatggatacaactatttggattggtatctgcagaagccaggccagtctccacacctcttgatctatttggcttctaatcgggcctccggggtccctgacaggttcagtggcagtggatcaggcacagattttacactgaaaatcagcagagtggaggctgaggatgttgggttttattactgcatgcaaactctacaaattccgctcactttcggcggagggaccaaggtggagatcaaa

SEQ ID NO: 205 - DNA, 351 bp, Artificial Sequence
  Description of Artificial Sequence: Synthetic polynucleotide
caggtgcagctgcaggagtcgggcccaggactggtgaagccttcggagaccctgtccctcacctgcgctgtctctggttactccgccagcggtgtttactactggggctggatccggcagcccccagggaaggggctggagtggattggaaatatctatcatagtgggagcacctattacaacccgtccctcgagaggcgagttagtatatcactagacacgtccaagaaccacttctccctgaggctgaattttgtgaccgccgcagacacggccgtgtattactgtgcgagagataggtttgatgcttttgatatctggggccaagggacaatggtcaccgtctcctca

SEQ ID NO: 206 - DNA, 321 bp, Artificial Sequence
  Description of Artificial Sequence: Synthetic polynucleotide
gaaatagtgatgacgcagtctccagccaccctgtctgtgtctccaggggaaagagccaccctctcctgcagggccagtcagagtattaacaacatcttagcctggtaccagcagaaacctggccaggctcccaggctcctcatctatggtgcatccaccagggccactggtatcccagccaggttcagtggcagtgggtctgggacagagttcactctcaccatcagcagcctgcagtctgaagattttgcagtttattactgtcagcagtataataactggcctctcactttcggcggagggaccaaggtggagatcaaa

SEQ ID NO: 207 - DNA, 363 bp, Artificial Sequence
  Description of Artificial Sequence: Synthetic polynucleotide
caggtgcagctggtggagtctgggggaggcgtggtccagcctgggaggtccctgagactctcctgtgcagcgtctggattcacctttaggagtcatggcatgcactgggtccgccaggctccaggcaagggactggagtgggtggcagttatatggtatgatggaagtagtgagtactatgcagactccgtgaagggccgattcaccatctccagagacaattccaagaacacgctgtatctgcaaatgaacagcctgagagccgaggacacggctgtgtattattgtgcgagagaaaacgtgtatggcagtggctggttttttgactactggggccagggaaccctggtcaccgtctcctca

SEQ ID NO: 208 - DNA, 324 bp, Artificial Sequence
  Description of Artificial Sequence: Synthetic polynucleotide
gaaatagtgatgacgcagtctccagccaccctgtctgtgtctccaggggaaagagcctccctctcctgcagggccagtcagagtgttggcagcaacttagcctggtaccagcagagacctggccaggctcccaggctcctcatctttggtgcatccaccagggccactggtatcccagccaggttcagtggcagtaggtctgggacagagttcactctcaccatcagcagcctgcagtctgaagattttgcactttattactgtcagcagtataataactggcctccgtggacgttcggccaagggaccaagctggagatcaaa

SEQ ID NO: 209 - DNA, 363 bp, Artificial Sequence
  Description of Artificial Sequence: Synthetic polynucleotide
caggtgcagctggtggagtctgggggaggcgtggtccagcctgggaggtccctgagactctcctgtgcagcgtctggattcaccttcaggagtcatggcatgcactgggtccgccaggcaccaggcaagggactggagtgggtggcagttatatggtatgatggaagtagtgactactatgcagactccgtgaagggccgattcaccatctccagagacaattccaagaacacactatttctgcaaatgaacagcctgagcgccgaggacacggctgtgtattattgtgcgagagaaaacgtgtatggcagtggctggttttttgactactggggccagggaaccctggtcaccgtctcctca

SEQ ID NO: 210 - DNA, 324 bp, Artificial Sequence
  Description of Artificial Sequence: Synthetic polynucleotide
gaaatagtgatgacgcagtctccagccaccctgtctgtgtctccaggggaaagagcctccctctcctgcagggccagtcagagtgttggcagcaacttagcctggtaccagcagaaacctggccaggctcccaggctcctcatctttggtgcatccaccagggccactggtatcccagccaggttcagtggcagtaggtctgggacagagttcactctcaccatcagcagcctgcagtctgaagattttgcactttattactgtcagcagtataataactggcctccgtggacgttcggccaagggaccaagctggagatcaaa

SEQ ID NO: 211 - DNA, 351 bp, Artificial Sequence
  Description of Artificial Sequence: Synthetic polynucleotide
gaggtgcagctgttggagtctgggggaggcttggtacagcctggggggtccctgagactctcctgtgcagcctctggattcacctttagcaactatgccatgacctgggtccgccaggctccagggaaggggctggagtgggtctcaagtattagtattagtcgtgctggcacatactacgcagactccgtgaagggccggttcaccatctccagagacaattccaagaacacgctgaatctgcaaatgaacagcctgagagccgaggacacggccgaatattactgtgcgagagagtactactacggcatggacgtctggggccaagggaccacggtcaccgtctcctca

SEQ ID NO: 212 - DNA, 321 bp, Artificial Sequence
  Description of Artificial Sequence: Synthetic polynucleotide
gaaattgtgttgacacagtctccagccaccctgtctttgtctccaggggaaagagccaccctctcctgcagggccagtcagagtgttagcagctacttagcctggtaccaacagaaacctggccagactcccaggctcctcatctatgatgcatccaacagggccactggcatcccagccaggttcagtggcagtgggtctgggacagacttcacgctcaccatcagcagcctagagactgaagattttgcagtttattactgtcagcagcttatcaactggccgctcactttcggcggagggaccaagctggagatcaaa

SEQ ID NO: 213 - DNA, 321 bp, Artificial Sequence
  Description of Artificial Sequence: Synthetic polynucleotide
gacatccagatgacccagtctccatcctccctgtctgcatctgtaggagacagagtcatcatcacttgccgggcgagtcaaggcattagcaattatttagcctggtttcagcagaaaccagggaaagctcctaacctcctgatctatgctgcatccactttgcgatcaggggtcccatctcggttcagtggcagtggatctgggacagatttcactctcaccatcagcagcctgcagcctgaagatgttgcaacttattactgtcaaaagtataacagtgccccgtacacttttggccaggggaccaaggtggagatcaaa

SEQ ID NO: 214 - DNA, 351 bp, Artificial Sequence
  Description of Artificial Sequence: Synthetic polynucleotide
gaggtgcagttgttggaatctggggcagacttggtacagcctggggggtccctgagactctcctgtgcagcctctggattcacctttagcagctatgccatgagttgggtccgccaggctccaggaaaggggctggagtgggtctcaactattcgtattagtggtggcaccacatactacgcagactccgtgaagggccggttcaccatctccagagacaattccaagaacacgctgtatctgcaaatgaacagcctgagagccgaagacacggccgtatattactgcgtaagggactactataacggtatggacgtctggggccaagggaccacggtcaccgtctcctca

SEQ ID NO: 215 - DNA, 321 bp, Artificial Sequence
  Description of Artificial Sequence: Synthetic polynucleotide
gaaattgtgttgacacagtctccagccaccctgtctttgtctccaggggaaagagccaccctctcctgcagggccagtcagcgtgttagcagctacttagcctggtaccaacagaaacctggccaggctcccaggctcctcatctatgatgcatccaacagggccactggcatcccagccaggttcagtggcagtgggtctgggacagacttcactctcaccatcagcagcctagagcctgaagattttgcagtttattactgtcagcagcgtagctactggcctcccgcttttggccaggggaccaagctggagatcaaa

SEQ ID NO: 216 - DNA, 261 bp, Artificial Sequence
  Description of Artificial Sequence: Synthetic polynucleotide
agctatgccatgagctgggtccgccaggctccagggaaggggctggagtgggtctcaagtattagtggtagtggtgatagcacaaactacgcagactccgtgaagggccggttcaccatctccagagacaattccaagaacacgctgcatctgcaaatgaacagcctgagagccgaggacacggccgtatattactgcgtaagggactactactacggtatggacgtctggggccacgggaccacggtcaccgtctcctca

SEQ ID NO: 217 - DNA, 321 bp, Artificial Sequence
  Description of Artificial Sequence: Synthetic polynucleotide
gaaattgtgttgacacagtctccagccaccctgtctttgtctccaggggaaagagccaccctctcctgcagggccagtcagagtgttaacagctacttagcctggtaccaacagaaacctggccaggctcccaggctcctcatctatgatgcatccaacagggccactggcatcccagccaggttcagtggcagtgggtctgggacagacttcactctcaccatcagcagcctagagcctgaagattttgcagtttattactgtcagcagcgtagctactggccgatcaccttcggccaagggacacgactggagattaaa

SEQ ID NO: 218 - DNA, 351 bp, Artificial Sequence
  Description of Artificial Sequence: Synthetic polynucleotide
gaggcgcagctgttggagtctgggggaggcttggtacagcctggggggtccctgagactctcctgtgcagcctctggattcacctttagcagctatgccatgagctgggtccgccaggctccagggaaggggctggagtgggtctcaactattagtggtagtggtggtagtacacactacgcagactccgtgaagggccggttcaccatctccagagacaattccaagaatacgttgtatctgcaaatgaacagcctgagagccgaggacacggccgtatattactgcgtaagggactactactacggtatggacgtctggggccaagggaccacggtcaccgtctcctca

SEQ ID NO: 219 - DNA, 321 bp, Artificial Sequence
  Description of Artificial Sequence: Synthetic polynucleotide
gaaattgtgttgacacagtctccagccaccctgtctttgtctccaggggaaagagccaccctctcctgcagggccagtcagagtgttagcagctacttagcctggtaccaacagaaacctggccaggctcccaggctcctcatctatgatgcatccaacagggccactggcatcccagccaggttcagtggcagtgggtctgggacagacttcactctcaccatcagcagcctagagcctgaagattttgcagtttattactgtcagcagcgtagctactggcctcccacttttggccaggggaccaagctggagatcaaa

SEQ ID NO: 220 - DNA, 363 bp, Artificial Sequence
  Description of Artificial Sequence: Synthetic polynucleotide
caggtgcagctggtggagtctgggggaggcgtggtccagcctgggaggtccctgagactctcctgtgcagcgtctggattcaccttcagtagctatggaatgcactgggtccgccaggctccaggcaaggggctggagtgggtggcagttatatggtatgatggaagtaaaaaatactatgtagactccgtgcagggccgattcaccatctccagagacaattccaagaatacgctgtatctgcaaatgaacagcctgagaggcgaggacacggctgtgtattactgtgcgagagatgggggagcagtggctgacaattggatcgactcctggggccagggaaccctggtcaccgtctcctca

SEQ ID NO: 221 - DNA, 321 bp, Artificial Sequence
  Description of Artificial Sequence: Synthetic polynucleotide
gacatccagatgacccagtctccatcctccctgtctgcgtctgtaggagacagagtcactctcacttgccgggcaagtcagaacattagaagctatttaaattggtatcagcagaaaccagggaaagcccctaagctcctgatctttgctgcatccagtttgccaagtggggtcccatcaaggttcagtggcagtggatctgtgacagatttcactctcaccgtcagcagtctgcaacctgaagattttgcaacttactcctgtcaacagagttacagtaccccgtacacttttggccaggggaccaagctggagatcaaa

SEQ ID NO: 222 - DNA, 351 bp, Artificial Sequence
  Description of Artificial Sequence: Synthetic polynucleotide
gaggaacagctgttggaatctggggcagacttggcacagccgggggggtccctgagactctcctgtgcagcctctggattcacctttagcagctatgccatgagttgggtccgccaggctccaggaaagggactggagtgggtctcaactattcgtattagtggtgataccacttactacgcagactccgtgaagggccggttcaccatctccagagacaattccaagaacacgctgtttctgcaaatgaacagcctgagagccgaagacacggccgtgtattactgcgtaagggactactataacggtatggacgtctggggccatgggaccacggtcaccgtctcctca

SEQ ID NO: 223 - DNA, 321 bp, Artificial Sequence
  Description of Artificial Sequence: Synthetic polynucleotide
gaaattgtgttgacacagtctccagccaccctgtctttgtctccaggggaaagagccaccctctcctgcagggccagtcagcgtgttagcagctatttagcctggtaccaacagaaacctggccaggctcccaggctcctcatctatgatgcatccaacagggccactggcatcccagccaggttcagtggcagtgggtctgggacagacttcactctcaccatcagcagcctagagcctgaagattttgcagtttattactgtcagcagcgtagctactggcctcccgcttttggccaggggaccaagctggagatcaaa

SEQ ID NO: 224 - DNA, 363 bp, Artificial Sequence
  Description of Artificial Sequence: Synthetic polynucleotide
caggtgcagctggtgcagtctggggctgaggtgaagaagcctggggcctcagtgaaggtctcctgcaaggcttctggatacaccttcaccggctactatatgcactgggtgcgacaggcccctggacaagggcttgagtggatgggatggatcaaccctaacagtggtggcacaaactatgcacagaagtttcagggcagggtcaccatgaccagggacacgtccatcagcacagcctacatggagctgagcaggctgagatctgacgacacggccgtgtattactgtgcgagagaagcagtggctggtacctctgatgcttttgatatctggggccaagggacaatggtcaccgtctcctca

SEQ ID NO: 225 - DNA, 321 bp, Artificial Sequence
  Description of Artificial Sequence: Synthetic polynucleotide
gacatccagatgacccagtctccatcctccctgtctgcatctgttggagacagagtcaccatcacttgccgggcaaatcagagtattgccagttatttaaattggtatcagcagaaaccaggaaaagtccctaaactcctgatctatggtgcatccagtttgcaaaatggggtcccatcaaggttcagtggcagtggatctaggacagatttcactctcaccatcagcagtctgcaacctgaagattttgcaacttactactgtcaacaaagttacagcaccgaaatcaccttcggccaagggacacgactggagattaaa

SEQ ID NO: 226 - DNA, 321 bp, Artificial Sequence
  Description of Artificial Sequence: Synthetic polynucleotide
gacatccagatgacccagtctccatcctccctgtctgcatctgtaggagacagagtcgccatcacttgccgggcaagtcagagtattgccagttatttaaattggtatcagcagaaaccagggaaagcccctaaactcctgatctatggtgcatccagtttgcaaaatggggtcccatcaaggttcagtggcagtggatctaggacagatttcactctcaccatcagcagtctgcaacctgaagattttgcaacttactactgtcaacagagttacagcaccgagatcaccttcggccaagggacacgactggagattaaa

SEQ ID NO: 227 - DNA, 360 bp, Artificial Sequence
  Description of Artificial Sequence: Synthetic polynucleotide
caggtgcagctggtggagtctgggggaggcgtggtccagcctgggaggtccctgcgactctcctgtgcagcgtctggattcacctttaggaactatggcatgcactgggtccgccaggctccaggcaaggggctggagtgggtggcagttatatggtatgatggaagtaataaattctatgcagactccgtgaagggccgattcaccatctccagagacaattccaagaacacgctgtatctgcaaatgaacagcctgagagtcgaggacacggctgtatattactgtgcgagagaggaggggatagcagtggccccctttgactactggggccagggaaccctggtcaccgtctcctca

SEQ ID NO: 228 - DNA, 321 bp, Artificial Sequence; identical to SEQ ID NO: 200
  Description of Artificial Sequence: Synthetic polynucleotide

SEQ ID NO: 229 - DNA, 363 bp, Artificial Sequence
  Description of Artificial Sequence: Synthetic polynucleotide
caggtgcagctggtggaatctgggggaggcatggtccagcctgggaggtccctgagactctcctgtacagcgtctggattcaccttcagtagtcatggcatgcactgggtccgccaggctccaggcaagggactggagtgggtggcagttatttggtttgatggaagtaatgaatattatgtagactccgtgaagggccgattcaccatctccagagacaattccaagaacacactgtatctgcaaatgaacagcctgagagccgaggacacggctgtgtattattgtgcgagagaaaacgtttatggcagtggctggttttttgactactggggccagggaaccctggtcaccgtctcctca

SEQ ID NO: 230 - DNA, 324 bp, Artificial Sequence
  Description of Artificial Sequence: Synthetic polynucleotide
gaaatagtgatgacgcagtctccagccaccctgtctgtgtctccaggggaaagagcctccctctcctgcagggccagtcagagtgttggcagcaacttagcctggtaccagcagaaacctggccaggctcccaggctcctcatctttggtgcatccaccagggccactggtatcccagccaggttcagtggcagtaggtctgggacagagttcactctcaccatcagcagcctgcagtctgaagattttgcactttattactgtcagcagtataataactggcctccgtggacgttcggccaagggaccaaggtggagatcaaa

SEQ ID NO: 231 - DNA, 363 bp, Artificial Sequence
  Description of Artificial Sequence: Synthetic polynucleotide
cagttgcagctggtggagtctgggggaggcgtggtccagcctggcaggtccctgagactctcctgtgcagcgtctggattcaccttcagtagttatggcatgcactgggtccgccaggctccaggcaagggactggagtgggtggcagttatatggtatgatggaagtagtgagtactatgcagactccgtgaagggccgattcaccatctccagagacaattccaagaacacgctgtatctgcaaatgaacagcctgagagccgaggacacggctgtgtattattgtgcgagagaaaacgtgtatggcagtggctggttttttgactactggggccagggaaccctggtcaccgtctcctca

SEQ ID NO: 232 - DNA, 324 bp, Artificial Sequence; identical to SEQ ID NO: 230
  Description of Artificial Sequence: Synthetic polynucleotide

SEQ ID NO: 233 - DNA, 272 bp, Artificial Sequence
  Description of Artificial Sequence: Synthetic polynucleotide
gtcatggcatgcactgggtccgccaggctccaggcaagggactggagtgggtggcagttatatggtatgatggaagtagtgagtactatgcagactccgtgaagggccgattcaccatctccagagacaattccaagaacacgctgtatctgcaaatgaacagcctgagagccgaggacacggctgtgtattattgtgcgagagaaaacgtatatggcagtggctggttttttgactactggggccagggaagcctggtcaccgtctcctca

SEQ ID NO: 234 - DNA, 324 bp, Artificial Sequence; identical to SEQ ID NO: 210
  Description of Artificial Sequence: Synthetic polynucleotide

SEQ ID NO: 235 - DNA, 363 bp, Artificial Sequence
  Description of Artificial Sequence: Synthetic polynucleotide
cagttgcagttggtggagtctgggggaggcgtggtccagtttggcaggtccctgagactctcctgtgcagcgtctggattcaccttcagtagtcatggcatgcactgggtccgccaggctccaggcaagggactggagtgggtggcagttatatggtatgatggaagtagtgagtactatgcagactccgtgaagggccgattcaccatctccagagacaattccaagaacacgctgtatctgcaaatgaacagcctgagagccgaggacacggctgtgtattattgtgcgagagaaaacgtgtatggcagtggctggttttttgactactggggccagggaaccctggtcaccgtctcctca

SEQ ID NO: 236 - DNA, 324 bp, Artificial Sequence; identical to SEQ ID NO: 210
  Description of Artificial Sequence: Synthetic polynucleotide

SEQ ID NO: 237 - DNA, 363 bp, Artificial Sequence
  Description of Artificial Sequence: Synthetic polynucleotide
cagttgcagctggtggagtctgggggaggcgtggtccagcctggcaggtccctaagactctcctgtgcagcgtctggattcaccttcagtagttatggcatgcactgggtccgccaggctccaggcaagggactggagtgggtggcagttatatggtatgatggaagtagtgagtattatgcagactccgtgaagggccgattcaccatctccagagacaattccaagaacacgctgtttctgcaaatgaacagcctgagagccgatgacacggctgtgtattattgtgcgagagaaaacgtgtatggcagtggctggttttttgactactggggccagggaaccctggtcaccgtctcctca

SEQ ID NO: 238 - DNA, 324 bp, Artificial Sequence
  Description of Artificial Sequence: Synthetic polynucleotide
gaaatagtgatgacgcagtctccagccaccctgtctgtgtctccaggggaaagagcctccctctcctgcagggccagtcagagtgttggcagcaacttagcctggtaccagcagaaacctggccaggctcccaggctcctcatctttggtgcatccaccagggccactggtatcccagccaggttcagtggcagtaggtctgggacagagttcactctcaccatcagcagcctgcagtctgaagattttgcactttattactgtcagcagtatgataactggcctccgtggacgttcggccaagggaccaagctggagatcaaa

SEQ ID NO: 239 - DNA, 363 bp, Artificial Sequence
  Description of Artificial Sequence: Synthetic polynucleotide
caggtgcagctggtggagtctgggggaggcgtggtccagcctgggaggtctctgagactctcctgtgcagcgtctggattcaccttaagtggctatggcatgcactgggtccgccaggctccaggcaagggactggagtgggtggcagttatatggtatgatggaagtaataaatactatgcagactccgtgaagggccgattcaccatctccagagacaattccaagaacatgctgtttctgcaaatgaacagcctgagagccgaggacacggctgtgtattactgtgtgagagaaaacgggtttggcagtggctggttttttgactactggggccagggaaacctggtcaccgtctcctca

SEQ ID NO: 240 - DNA, 324 bp, Artificial Sequence
  Description of Artificial Sequence: Synthetic polynucleotide
gaaatagtgatgacgcagtctccagccaccctgtctgtgtctccaggggaaagagccaccctctcctgcaggaccagtcagagtgtaagtagagacttagcctggtaccagcagaaacctggccaggctcccaggctcctcatctatggtgcatccaccagggccactggtattccagtcaggttcagtggcagtgggtctgggacagagttcactctcaccatcagcagcctgcagtctgaagattttgcagtttattactgtcagcagtataataactggcctccgtggacgttcggccaagggaccaagctggagatcaaa

SEQ ID NO: 241 - DNA, 375 bp, Artificial Sequence
  Description of Artificial Sequence: Synthetic polynucleotide
caggggcagctggtggagtctgggggaggcgtggtccagcctgggaggtccctgagactctcctgtgcagcgtctggattcaccttcagtagttataccttgcactgggtccgccaggctccaggcaaggggctggagtgggtggcagtcatatggtatgatggaagtaataagtattatgtagactccgtgaagggccgattcaccatctccagagacaattccaagaacacgctgtatctgcaaatgaacagcctgagagccgaggacacggctgtgtattactgtgcgagagagtatggttcggggagttattataacgtctactacggtatggacgtctggggccaggggaccacggtcaccgtctcctca

SEQ ID NO: 242 - DNA, 336 bp, Artificial Sequence
  Description of Artificial Sequence: Synthetic polynucleotide
gatattgtgatgactcagtctccactctccctgcccgtcacccctggagagccggcctccatctcctgcaggtctagtcagagcctcctgcatagcaatggatacaagtatttggattggtatctgcagaaagcagggcagtctccacacctcttgatctatttgggttctaatcgggcctccggggtccctgacaggttcagtggcagtggatcaggcacagattttacactgaaaatcagcagagtggaggctgaggatgttggattttattactgcatgcaaactctacaaattccgctcactttcggcggagggaccaagctggagatcaaa

SEQ ID NO: 243 - DNA, 360 bp, Artificial Sequence
  Description of Artificial Sequence: Synthetic polynucleotide
gaggtgcaggtggtggagtctgggggaggcttggtccagcctggggggtccctgagactctcctgtgcaacctctggattcacctttagaagctattggatgacctgggtccgccaggctccagggaaggggctggagtgggtggccaatataaagcaggatggaagtgagagacactatgtggactctgtgaagggccgattcaccatctccagagacaacgccaagacatcactgtatctgcaaatgagcagcctgagagccgaggacacggctatgtattactgtgcgagagaggggtactatggttcgggctactttgactactggggccagggaaccctggtcaccgtctcctca

SEQ ID NO: 244 - DNA, 321 bp, Artificial Sequence
  Description of Artificial Sequence: Synthetic polynucleotide
gacatccagatgacccagtctccctccaccctgtctgcatctgtaggagacagagtcatcatcacttgccgggccagtcagagtattagtagggggttggcctggtatcagcagaaaccagggaaagcccctaaactcttgatctataaggcgtctaatttagaaagtggggtcccatcaaggttcagcggcagtggatctgggacagaattcactctcaccatcagcagcctgcagcctgatgattttgcagcttattactgccaacagtatagttattattctcacacttttggccaggggaccaaggtggagatcaaa

SEQ ID NO: 245 - DNA, 360 bp, Artificial Sequence
  Description of Artificial Sequence: Synthetic polynucleotide
gaggtgcaactggtggagtctgggggaggcttggtccagcctggggggtccctgagactctcctgtgcagcctctggattcaccttaagtttctattggatgacctgggtccgccaggctccagggaaggggctggagtgggtggccaacataaagcaagatggaaatgagaaaaactatgtggactctgtgaagggccgattcaccatctccaaagacaacgccaagaaatcagtgtttctgcaaatgaacagcctgagagccgaggacacggctgtgtattactgtgcgagagaggggtactttggttcgggctactttgactactggggccagggaaccctggtcaccgtctcctca

SEQ ID NO: 246 - DNA, 321 bp, Artificial Sequence
  Description of Artificial Sequence: Synthetic polynucleotide
gacatccagatgacccagtctccttccaccctgtctgcatctgtgggagacagagtcaccatcacttgtcgggccagtcagagtattaatagctggttggcctggtatcagcagaaaccagggaaagcccctaagctcctgatctataaggcgtctactttagaaagtggggtcccatcaaggttcagcggcagtggatctgggacagaattcactctcaccatcagcagcctgcagcctgatgattttgcaccttattactgccagcattataatagttatcctcacacttttggccaggggaccaaggtggagatcaaa

SEQ ID NO: 247 - DNA, 360 bp, Artificial Sequence
  Description of Artificial Sequence: Synthetic polynucleotide
gaggtgcagctggtggagtctgggggaggcttggtccagcctggggggtccctgagactctcctgtgcagcctctggattcacttttagtagttattggatgagctgggtccgccaggctccagggaaggggctggagtgggtggccaacataaagcaagatggaagtgagaaacactatgtggactctgtgaagggccgattcaccatctccagagacaacgccaagaactcactgtatctgcaaatgaacagcctgagagccgaggacacggctgtgtattactgtgcgagagaggggtactttggttcgggctactttgactactggggccagggaaccctggtcaccgtctcctca

SEQ ID NO: 248 - DNA, 321 bp, Artificial Sequence
  Description of Artificial Sequence: Synthetic polynucleotide
gacatccagttgacccagtctccatccttcctgtctgcatctgtaggagacagagtcaccatcacttgccgggccagtcagggcattagcagttatttagcctggtatcagcaaaaaccagggaaagcccctaagctcctgatctatgctgcatccactttgcaaagtggggtcccatcaaggttcagcggcagtggatctgggacagaattcactctcacaatcagcagcctgcagcctgaagattttgcaacttattactgccaacagtatagtttttattctcacacttttggccaggggaccaagctggagatcaaa

SEQ ID NO: 249 - DNA, 360 bp, Artificial Sequence
  Description of Artificial Sequence: Synthetic polynucleotide
gaggtgcaactggtggagtctgggggaggcttggtccagcctggggggtccctgagactctcctgtgcagcctctggattcaccttaagtttctattggatgacctgggtccgccaggctccagggaaggggctggagtgggtggccaatataaagcaagatggaaatgagaaaaactttgtggactctgtgaagggccgattcaccatctccagagacaacgccaagaaatcagtgtttctgcaaatgaacagcctgagagccgaggacacggctgtgtattactgtgcgagagaggggtactttggttcgggctactttgactactggggccagggaaccctggtcaccgtctcctca

SEQ ID NO: 250 - DNA, 321 bp, Artificial Sequence
  Description of Artificial Sequence: Synthetic polynucleotide
gacatccagatgacccagtctccttccaccctgtctgcatctgtaggagacagagtcaccatcacttgccgggccagtcagagtattaatagctggttggcctggtatcagcagaaaccagggaaagcccctaagctcctgatctataaggcgtctagtttagaaagtggggtcccatcaaggttcagcggcagtggatctgggacagaattcactctcaccatcagcagcctgcagcctgatgattttgcaacttattactgccagcagtataatagttatcctcacacttttggccaggggaccaagctggagatcaaa

SEQ ID NO: 251 - DNA, 321 bp, Artificial Sequence
  Description of Artificial Sequence: Synthetic polynucleotide
gacatccagttgacccagtctccatccttcctgtctgcatctgtaggagacagagtcaccatctcttgccgggccagtcagggcattagcagttatttggcctggtatcagcaaaaaccagggaaagcccctaagctcctgatctatgctgcatccactttgcaaggtggggtcccatcaaggttcagcggcagtggatctgggacaacattcactctcacaatcagcagcctgcagcctgaagattttgcaacttattactgtcaacagcttaatacttacccattcactttcggccctgggaccaagctggagatcaaa

SEQ ID NO: 252 - DNA, 321 bp, Artificial Sequence; identical to SEQ ID NO: 251
  Description of Artificial Sequence: Synthetic polynucleotide

SEQ ID NO: 253 - DNA, 357 bp, Artificial Sequence
  Description of Artificial Sequence: Synthetic polynucleotide
caggtgcagctgcaggagtcgggcccaggactggtgaagcctttggggaccctgtccctcacctgcgctgtctctggtggctccatcagcaatagtaactggtggagttgggtccgccagcccccaggaaaggggctggagtggattggagaaatctatcatagtgggagcaccaactacaacccgtccctcaagagtcgagtcaccatagcactagactggtccaagaaccagttctccctgcagctgaggtctgtgaccgccgcggacacggccgtgtattactgtgcgcggtatggttcgggtccttttggcggtgactactggggccagggaaccctggtcaccgtctcctca

SEQ ID NO: 254 - DNA, 369 bp, Artificial Sequence
  Description of Artificial Sequence: Synthetic polynucleotide
caggtgcagataaaggagtcgggcccaggactggtgaagccttcggagaccctgtccctcacctgcgctgtctctggtttctccttcagcagtggttattactggggctggatccggcagcccccagggaagggtctggagtggcttgggagtttctttcataatgggaatacctactacaacccgtccctcaggagtcgagtcaccatctcagtagacacgtccaagaaccacttctccctgaagctgacctctgtgaccgccgcagacacggccgtgtattactgtgcgggattcggggacttaccccattatcattattacgttatggacgtctggggccaagggaccacggtcaccgtctcctca

SEQ ID NO: 255 - DNA, 324 bp, Artificial Sequence
  Description of Artificial Sequence: Synthetic polynucleotide
gaaattgtgttgacacagtctccagccaccctgtctttgtctccaggggaaagagccaccctctcctgcagggccagtcagagtgttagcagctacttagcctggtaccaacagaaacctggccaggctcccaggctcctcatctatgatgcatccaacagggccattggcatcccagccaggttcagtggcagtgggtctgggacagacttcactctcaccatcagcagcctagagcctgaagattttgcagtttattactgtcagcagcgtagcaactggcctccgtacacttttggccaggggaccaagctggagatcaaa

SEQ ID NO: 256 - DNA, 369 bp, Artificial Sequence
  Description of Artificial Sequence: Synthetic polynucleotide
caggtgcagccaaaggagtcgggcccaggagtggtgaagccttcggagaccctgtccctcacctgcgctgtctctggtttccccatcagccgtggttattactggggctggatccggcagcccccagggaagggtctggagtggattgggaatatctttcatagtgggaccacctactacaatccgtccctcaagagtcgagtcaccatctcagtagacacgtccaagaaccagatctccctgaagctgacctctgtgaccgccgcagacacggccgtatattattgtgtgggattcggggacttgccccactaccaatattacgttatggacatctggggccaagggaccacggtcaccgtctcctca

SEQ ID NO: 257 - DNA, 324 bp, Artificial Sequence
  Description of Artificial Sequence: Synthetic polynucleotide
gaaattgtgttgacacagtctccagccaccctgtctttgtctccaggggaaagagccaccctctcctgcagggccagtcagagtgttagcagctacttagcctggtaccaacagaaacctggccaggctcccaggctcctcatctatgatgcatccaacagggccactggcatcccagccaggttcagtggcagtgggtctgggacagacttcactctcaccatcagcagcctagagcctgaagattttgcagtttattactgtcagcagcgtagcaactggcctccgtacacttttggccaggggaccaagctggagatcaaa

SEQ ID NO: 258 - DNA, 351 bp, Artificial Sequence
  Description of Artificial Sequence: Synthetic polynucleotide
caggtgcagctgcaggagtcgggcccaggactggtgaagccttcggagaccctgtccctcacctgcgctgtctctggttactccgccagcggtctttactactgggcctggatccggcagcccccagggaagggactggagtggattggaaatatctatcatagtgggagaacctactacaatccgtccctcgagagtcgagtcagcatatcactagacacgtccaagcaccaggtctccctgaaactgaaatctgtgacctacgcagacacggccgtgtatttctgtgcgagagataggtttgatggttttgatatttggggccaagggacaatggtcaccgtctcctca

SEQ ID NO: 259 - DNA, 321 bp, Artificial Sequence
  Description of Artificial Sequence: Synthetic polynucleotide
gaaatagtgatgacgcagtctccagccaccctgtctgtgtctccaggggaaagagccaccctctcctgcagggccagtcagactattaacaacatcttagcctggtaccagcagaaacctggccaggctcccaggctcctcatctatggtgcatccaccagggccactggtatcccagccaggttcagtggcagtgggtctgggacagagttcactctcaccatcagcagcctgcagtctgaagattttgcagtttattactgtcagcagtataataactggcctctcactttcggcggagggaccaagctggagatcaaa

SEQ ID NO: 260 - DNA, 40 bp, Artificial Sequence
  Description of Artificial Sequence: Synthetic oligonucleotide
atagctcttcagggaccatgaarcayctgtggttcttcct

SEQ ID NO: 261 - DNA, 39 bp, Artificial Sequence
  Description of Artificial Sequence: Synthetic oligonucleotide
atagctcttcagggaccatggacatactttgttccacgc

SEQ ID NO: 262 - DNA, 39 bp, Artificial Sequence
  Description of Artificial Sequence: Synthetic oligonucleotide
atagctcttcagggaccatggacacactttgctacacac

SEQ ID NO: 263 - DNA, 39 bp, Artificial Sequence
  Description of Artificial Sequence: Synthetic oligonucleotide
atagctcttcagggaccatgtctgtctccttcctcatct

SEQ ID NO: 264 - DNA, 38 bp, Artificial Sequence
  Description of Artificial Sequence: Synthetic oligonucleotide
atagctcttcagggaccatggactggacctggagvatc

SEQ ID NO: 265 - DNA, 38 bp, Artificial Sequence
  Description of Artificial Sequence: Synthetic oligonucleotide
atagctcttcagggaccatggactggatttggaggrtc

SEQ ID NO: 266 - DNA, 38 bp, Artificial Sequence
  Description of Artificial Sequence: Synthetic oligonucleotide
atagctcttcagggaccatggactgcacctggaggatc

SEQ ID NO: 267 - DNA, 38 bp, Artificial Sequence
  Description of Artificial Sequence: Synthetic oligonucleotide
atagctcttcagggaccatggactggacctggaggktc

SEQ ID NO: 268 - DNA, 38 bp, Artificial Sequence
  Description of Artificial Sequence: Synthetic oligonucleotide
atagctcttcagggaccatggagttkggrctgagctgg

SEQ ID NO: 269 - DNA, 38 bp, Artificial Sequence
  Description of Artificial Sequence: Synthetic oligonucleotide
atagctcttcagggaccatggagtttkggctkagctgg

SEQ ID NO: 270 - DNA, 38 bp, Artificial Sequence
  Description of Artificial Sequence: Synthetic oligonucleotide
atagctcttcagggaccatggaactggggctccgctgg

SEQ ID NO: 271 - DNA, 38 bp, Artificial Sequence
  Description of Artificial Sequence: Synthetic oligonucleotide
atagctcttcagggaccatggarttggggctgwgctgg

SEQ ID NO: 272 - DNA, 38 bp, Artificial Sequence
  Description of Artificial Sequence: Synthetic oligonucleotide
atagctcttcagggaccatggggtcaaccgccatcctc

SEQ ID NO: 273 - DNA, 44 bp, Artificial Sequence
  Description of Artificial Sequence: Synthetic oligonucleotide
atagctcttcagggaccatggacatgagggtsccygctcagctc

SEQ ID NO: 274 - DNA, 44 bp, Artificial Sequence
  Description of Artificial Sequence: Synthetic oligonucleotide
atagctcttcagggaccatggacatgagrgtcctcgctcagctc

SEQ ID NO: 275 - DNA, 41 bp, Artificial Sequence
  Description of Artificial Sequence: Synthetic oligonucleotide
atagctcttcagggaccatggaagccccagcdcagcttctc

SEQ ID NO: 276 - DNA, 41 bp, Artificial Sequence
  Description of Artificial Sequence: Synthetic oligonucleotide
atagctcttcagggaccatggaaaccccagcgcagcttctc

SEQ ID NO: 277 - DNA, 41 bp, Artificial Sequence
  Description of Artificial Sequence: Synthetic oligonucleotide
atagctcttcagggaccatggtgttgcagacccaggtcttc

SEQ ID NO: 278 - DNA, 41 bp, Artificial Sequence
  Description of Artificial Sequence: Synthetic oligonucleotide
atagctcttcagggaccatggggtcccaggttcacctcctc

SEQ ID NO: 279 - DNA, 41 bp, Artificial Sequence
  Description of Artificial Sequence: Synthetic oligonucleotide
atagctcttcagggaccatgaggctccytgctcagctcctg

SEQ ID NO: 280 - DNA, 33 bp, Artificial Sequence
  Description of Artificial Sequence: Synthetic oligonucleotide
atagctcttcttcgtttgatctccascttggtc

SEQ ID NO: 281 - DNA, 33 bp, Artificial Sequence
  Description of Artificial Sequence: Synthetic oligonucleotide
atagctcttcttcgtttaatctccagtcgtgtc

SEQ ID NO: 282 - DNA, 30 bp, Artificial Sequence
  Description of Artificial Sequence: Synthetic oligonucleotide
atagctcttctggctgaggagacggtgacc

SEQ ID NO: 283 - DNA, 34 bp, Artificial Sequence
  Description of Artificial Sequence: Synthetic oligonucleotide
atagctcttcatgtgacgctgttgtgactcagga

SEQ ID NO: 284 - DNA, 34 bp, Artificial Sequence
  Description of Artificial Sequence: Synthetic oligonucleotide
atagctcttcatgtgaccytgtgctcactcagtc

SEQ ID NO: 285 - DNA, 37 bp, Artificial Sequence
  Description of Artificial Sequence: Synthetic oligonucleotide
gatgctcttctgggctggcctaggacagtcamcytgg

SEQ ID NO: 286 - protein, 570 aa, Homo sapiens
MTLLWCVVSLYFYGILQSDASERCDDWGLDTMRQIQVFEDEPARIKCPLFEHFLKFNYSTAHSAGLTLIWYWTRQDRDLEEPINFRLPENRISKEKDVLWFRPTLLNDTGNYTCMLRNTTYCSKVAFPLEVVQKDSCFNSPMKLPVHKLYIEYGIQRITCPNVDGYFPSSVKPTITWYMGCYKIQNFNNVIPEGMNLSFLIALISNNGNYTCVVTYPENGRTFHLTRTLTVKVVGSPKNAVPPVIHSPNDHVVYEKEPGEELLIPCTVYFSFLMDSRNEVWWTIDGKKPDDITIDVTINESISHSRTEDETRTQILSIKKVTSEDLKRSYVCHARSAKGEVAKAAKVKQKVPAPRYTVELACGFGATVLLVVILIVVYHVYWLEMVLFYRAHFGTDETILDGKEYDIYVSYARNAEEEEFVLLTLRGVLENEFGYKLCIFDRDSLPGGIVTDETLSFIQKSRRLLVVLSPNYVLQGTQALLELKAGLENMASRGNINVILVQYKAVKETKVKELKRAKTVLTVIKWKGEKSKYPQGRFWKQLQVAMPVKKSPRRSSSDEQGLSYSSLKNV